European Patent Specification EP 4 121 110 B1, published May 27, 2026. Title: ANTI-CERAMIDE ANTIBODIES. Applicant: Ceramedix Holding, LLC Memorial Sloan-Kettering Cancer Center. The sequence listing filed with the application follows.

SEQUENCE LISTING (76 sequences)

SEQ ID NO: 1 - protein, 10 aa, Artificial Sequence
  HCDR1-IH
GYTFTDHTIH

SEQ ID NO: 2 - protein, 10 aa, Artificial Sequence
  HCDR1-IH-MH
GYTFTDHTMH

SEQ ID NO: 3 - protein, 17 aa, Artificial Sequence
  HCDR2-DG
YNYPRDGSTKYNEKFQG

SEQ ID NO: 4 - protein, 17 aa, Artificial Sequence
  HCDR2-DG-EG
YNYPREGSTKYNEKFQG

SEQ ID NO: 5 - protein, 17 aa, Artificial Sequence
  HCDR2-DG-DV
YNYPRDVSTKYNEKFQG

SEQ ID NO: 6 - protein, 17 aa, Artificial Sequence
  HCDR2-NE-AE
YNYPRDGSTKYAEKFQG

SEQ ID NO: 7 - protein, 11 aa, Artificial Sequence
  HCDR3
GFITTVVPSAY

SEQ ID NO: 8 - protein, 11 aa, Artificial Sequence
  LCDR1
RASKSISKYLA

SEQ ID NO: 9 - protein, 7 aa, Artificial Sequence
  LCDR2
SGSTLQS

SEQ ID NO: 10 - protein, 9 aa, Artificial Sequence
  LCDR3
QQHNEYPWT

SEQ ID NO: 11 - protein, 10 aa, Mus musculus
GYTFTDHTIH

SEQ ID NO: 12 - protein, 17 aa, Mus musculus
YNYPRDGSTKYNEKFKG

SEQ ID NO: 13 - protein, 11 aa, Mus musculus
GFITTVVPSAY

SEQ ID NO: 14 - protein, 11 aa, Mus musculus
RASKSISKYLA

SEQ ID NO: 15 - protein, 7 aa, Mus musculus
SGSTLQS

SEQ ID NO: 16 - protein, 9 aa, Mus musculus
QQHNEYPWT

SEQ ID NO: 17 - protein, 120 aa, Artificial Sequence
  Humanized VH1
QVQLVQSGAEVKKPGASVKVSCKASGYTFTDHTMHWVRQAPGQGLEWMGYNYPRDGSTKYAEKFQGRVTMTADKSTSTVYMELSSLRSEDTAVYYCAKGFITTVVPSAYWGQGTLVTVSS

SEQ ID NO: 18 - protein, 120 aa, Artificial Sequence
  Humanized VH2
QVQLVQSGAEVKKPGASVKVSCKVSGYTFTDHTIHWMRQAPGQGLEWMGYNYPRDGSTKYNEKFQGRVTMTADKSTSTVYMELSSLRSEDTAVYYCAKGFITTVVPSAYWGQGTLVTVSS

SEQ ID NO: 19 - protein, 120 aa, Artificial Sequence
  Humanized VH3
QVQLVQSGAEVKKPGATVKISCKVSGYTFTDHTIHWMQQAPGKGLEWMGYNYPRDGSTKYNEKFQGRVTITADKSTSTAYMELSSLRSEDTAVYYCAKGFITTVVPSAYWGQGTLVTVSS

SEQ ID NO: 20 - protein, 120 aa, Artificial Sequence
  Humanized VH4
QVQLVQSGAEVKKPGASVKVSCKVSGYTFTDHTIHWMRQAPGQGLEWMGYNYPREGSTKYNEKFQGRVTMTADKSTSTVYMELSSLRSEDTAVYYCAKGFITTVVPSAYWGQGTLVTVSS

SEQ ID NO: 21 - protein, 120 aa, Artificial Sequence
  Humanized VH5
QVQLVQSGAEVKKPGASVKVSCKVSGYTFTDHTIHWMRQAPGQGLEWMGYNYPRDVSTKYNEKFQGRVTMTADKSTSTVYMELSSLRSEDTAVYYCAKGFITTVVPSAYWGQGTLVTVSS

SEQ ID NO: 22 - protein, 107 aa, Artificial Sequence
  Humanized VL1
DIQLTQSPSFLSASVGDRVTITCRASKSISKYLAWYQQKPGKAPKLLIYSGSTLQSGVPSRFSGSGSGTEFTLTISSLQPEDFATYYCQQHNEYPWTFGGGTKVEIK

SEQ ID NO: 23 - protein, 107 aa, Artificial Sequence
  Humanized VL2
DVQITQSPSFLSASVGDRVTITCRASKSISKYLAWYQQKPGKANKLLIYSGSTLQSGVPSRFSGSGSGTDFTLTISSLQPEDFATYYCQQHNEYPWTFGGGTKVEIK

SEQ ID NO: 24 - protein, 107 aa, Artificial Sequence
  Humanized VL3
DVQLTQSPSSVSASVGDRVTITCRASKSISKYLAWYQQKPGKAPKLLIYSGSTLQSGVPSRFSGSGSGTDFTLTISSLQPEDFATYYCQQHNEYPWTFGPGTKVEIK

SEQ ID NO: 25 - protein, 20 aa, Artificial Sequence
  STD1 linker
NYGGGGSGGGGSGGGGSGNS

SEQ ID NO: 26 - protein, 38 aa, Artificial Sequence
  STD2 linker
NYGGGGSGGGGSGGGGSGNYGGGGSGGGGSGGGGSGNS

SEQ ID NO: 27 - protein, 2 aa, Artificial Sequence
  H1 linker
NS

SEQ ID NO: 28 - protein, 8 aa, Artificial Sequence
  H2 linker
GGGGSGNS

SEQ ID NO: 29 - protein, 10 aa, Artificial Sequence
  H3 linker
NYGGGGSGNS

SEQ ID NO: 30 - protein, 13 aa, Artificial Sequence
  H4 linker
GGGGSGGGGSGNS

SEQ ID NO: 31 - protein, 15 aa, Artificial Sequence
  H5 linker
NYGGGGSGGGGSGNS

SEQ ID NO: 32 - protein, 18 aa, Artificial Sequence
  H6 linker
GGGGSGGGGSGGGGSGNS

SEQ ID NO: 33 - protein, 8 aa, Artificial Sequence
  H7 linker
GCPPCPNS

SEQ ID NO: 34 - protein, 5 aa, Artificial Sequence
  Gly4Ser linker
GGGGS

SEQ ID NO: 35 - protein, 15 aa, Artificial Sequence
  (G4S)3 linker
GGGGSGGGGSGGGGS

SEQ ID NO: 36 - protein, 16 aa, Artificial Sequence
  H105 linker
SGGGGSGGGGSGGGGS

SEQ ID NO: 37 - protein, 20 aa, Artificial Sequence
  (G4S)4 linker
GGGGSGGGGSGGGGSGGGGS

SEQ ID NO: 38 - protein, 21 aa, Artificial Sequence
  H75 linker (NKG2A quadruple mutant)
QRHNNSSLNTGTQMAGHSPNS

SEQ ID NO: 39 - protein, 16 aa, Artificial Sequence
  H83 linker (NKG2A derived)
SSLNTGTQMAGHSPNS

SEQ ID NO: 40 - protein, 18 aa, Artificial Sequence
  H106 linker (NKG2A derived)
QRHNNSSLNTGTQMAGHS

SEQ ID NO: 41 - protein, 14 aa, Artificial Sequence
  H81 linker (NKG2D derived)
EVQIPLTESYSPNS

SEQ ID NO: 42 - protein, 20 aa, Artificial Sequence
  H91 linker (NKG2D derived)
NSLANQEVQIPLTESYSPNS

SEQ ID NO: 43 - protein, 19 aa, Artificial Sequence
  H94 linker
SGGGGSGGGGSGGGGSPNS

SEQ ID NO: 44 - protein, 19 aa, Artificial Sequence
  H111 linker
SGGGGSGGGGSGGGGSPGS

SEQ ID NO: 45 - protein, 19 aa, Artificial Sequence
  H113 linker
SGGGGSGGGGSGGGGSPAS

SEQ ID NO: 46 - protein, 18 aa, Artificial Sequence
  H114 linker
SGGGGSGGGGSGGGGSPS

SEQ ID NO: 47 - protein, 19 aa, Artificial Sequence
  H115 linker
SGGGGSGGGGSGGGGSPSS

SEQ ID NO: 48 - protein, 283 aa, Artificial Sequence
  VH2-VL1 (Lead) scFv
MEWSWVFLFFLSVTTGVHSQVQLVQSGAEVKKPGASVKVSCKVSGYTFTDHTIHWMRQAPGQGLEWMGYNYPRDGSTKYNEKFQGRVTMTADKSTSTVYMELSSLRSEDTAVYYCAKGFITTVVPSAYWGQGTLVTVSSGGGGSGGGGSGGGGSDIQLTQSPSFLSASVGDRVTITCRASKSISKYLAWYQQKPGKAPKLLIYSGSTLQSGVPSRFSGSGSGTEFTLTISSLQPEDFATYYCQQHNEYPWTFGGGTKVEIKRAAAGGGGSGGGGSHHHHHHHH

SEQ ID NO: 49 - protein, 283 aa, Artificial Sequence
  VH4-VL1 scFv
MEWSWVFLFFLSVTTGVHSQVQLVQSGAEVKKPGASVKVSCKVSGYTFTDHTIHWMRQAPGQGLEWMGYNYPREGSTKYNEKFQGRVTMTADKSTSTVYMELSSLRSEDTAVYYCAKGFITTVVPSAYWGQGTLVTVSSGGGGSGGGGSGGGGSDIQLTQSPSFLSASVGDRVTITCRASKSISKYLAWYQQKPGKAPKLLIYSGSTLQSGVPSRFSGSGSGTEFTLTISSLQPEDFATYYCQQHNEYPWTFGGGTKVEIKRAAAGGGGSGGGGSHHHHHHHH

SEQ ID NO: 50 - protein, 283 aa, Artificial Sequence
  VH5-VL1 scFv
MEWSWVFLFFLSVTTGVHSQVQLVQSGAEVKKPGASVKVSCKVSGYTFTDHTIHWMRQAPGQGLEWMGYNYPRDVSTKYNEKFQGRVTMTADKSTSTVYMELSSLRSEDTAVYYCAKGFITTVVPSAYWGQGTLVTVSSGGGGSGGGGSGGGGSDIQLTQSPSFLSASVGDRVTITCRASKSISKYLAWYQQKPGKAPKLLIYSGSTLQSGVPSRFSGSGSGTEFTLTISSLQPEDFATYYCQQHNEYPWTFGGGTKVEIKRAAAGGGGSGGGGSHHHHHHHH

SEQ ID NO: 51 - protein, 264 aa, Artificial Sequence
  VH2-VL1 scFv - no signal sequence
QVQLVQSGAEVKKPGASVKVSCKVSGYTFTDHTIHWMRQAPGQGLEWMGYNYPRDGSTKYNEKFQGRVTMTADKSTSTVYMELSSLRSEDTAVYYCAKGFITTVVPSAYWGQGTLVTVSSGGGGSGGGGSGGGGSDIQLTQSPSFLSASVGDRVTITCRASKSISKYLAWYQQKPGKAPKLLIYSGSTLQSGVPSRFSGSGSGTEFTLTISSLQPEDFATYYCQQHNEYPWTFGGGTKVEIKRAAAGGGGSGGGGSHHHHHHHH

SEQ ID NO: 52 - protein, 264 aa, Artificial Sequence
  VH4-VL1 scFv - no signal sequence
QVQLVQSGAEVKKPGASVKVSCKVSGYTFTDHTIHWMRQAPGQGLEWMGYNYPREGSTKYNEKFQGRVTMTADKSTSTVYMELSSLRSEDTAVYYCAKGFITTVVPSAYWGQGTLVTVSSGGGGSGGGGSGGGGSDIQLTQSPSFLSASVGDRVTITCRASKSISKYLAWYQQKPGKAPKLLIYSGSTLQSGVPSRFSGSGSGTEFTLTISSLQPEDFATYYCQQHNEYPWTFGGGTKVEIKRAAAGGGGSGGGGSHHHHHHHH

SEQ ID NO: 53 - protein, 264 aa, Artificial Sequence
  VH5-VL1 scFv - no signal sequence
QVQLVQSGAEVKKPGASVKVSCKVSGYTFTDHTIHWMRQAPGQGLEWMGYNYPRDVSTKYNEKFQGRVTMTADKSTSTVYMELSSLRSEDTAVYYCAKGFITTVVPSAYWGQGTLVTVSSGGGGSGGGGSGGGGSDIQLTQSPSFLSASVGDRVTITCRASKSISKYLAWYQQKPGKAPKLLIYSGSTLQSGVPSRFSGSGSGTEFTLTISSLQPEDFATYYCQQHNEYPWTFGGGTKVEIKRAAAGGGGSGGGGSHHHHHHHH

SEQ ID NO: 54 - protein, 264 aa, Artificial Sequence
  VH1-VL1 scFv
QVQLVQSGAEVKKPGASVKVSCKASGYTFTDHTMHWVRQAPGQGLEWMGYNYPRDGSTKYAEKFQGRVTMTADKSTSTVYMELSSLRSEDTAVYYCAKGFITTVVPSAYWGQGTLVTVSSGGGGSGGGGSGGGGSDIQLTQSPSFLSASVGDRVTITCRASKSISKYLAWYQQKPGKAPKLLIYSGSTLQSGVPSRFSGSGSGTEFTLTISSLQPEDFATYYCQQHNEYPWTFGGGTKVEIKRAAAGGGGSGGGGSHHHHHHHH

SEQ ID NO: 55 - protein, 264 aa, Artificial Sequence
  VH1-VL2 scFv
QVQLVQSGAEVKKPGASVKVSCKASGYTFTDHTMHWVRQAPGQGLEWMGYNYPRDGSTKYAEKFQGRVTMTADKSTSTVYMELSSLRSEDTAVYYCAKGFITTVVPSAYWGQGTLVTVSSGGGGSGGGGSGGGGSDVQITQSPSFLSASVGDRVTITCRASKSISKYLAWYQQKPGKANKLLIYSGSTLQSGVPSRFSGSGSGTDFTLTISSLQPEDFATYYCQQHNEYPWTFGGGTKVEIKRAAAGGGGSGGGGSHHHHHHHH

SEQ ID NO: 56 - protein, 264 aa, Artificial Sequence
  VH1-VL3 scFv
QVQLVQSGAEVKKPGASVKVSCKASGYTFTDHTMHWVRQAPGQGLEWMGYNYPRDGSTKYAEKFQGRVTMTADKSTSTVYMELSSLRSEDTAVYYCAKGFITTVVPSAYWGQGTLVTVSSGGGGSGGGGSGGGGSDVQLTQSPSSVSASVGDRVTITCRASKSISKYLAWYQQKPGKAPKLLIYSGSTLQSGVPSRFSGSGSGTDFTLTISSLQPEDFATYYCQQHNEYPWTFGPGTKVEIKRAAAGGGGSGGGGSHHHHHHHH

SEQ ID NO: 57 - protein, 264 aa, Artificial Sequence
  VH2-VL2 scFv
QVQLVQSGAEVKKPGASVKVSCKVSGYTFTDHTIHWMRQAPGQGLEWMGYNYPRDGSTKYNEKFQGRVTMTADKSTSTVYMELSSLRSEDTAVYYCAKGFITTVVPSAYWGQGTLVTVSSGGGGSGGGGSGGGGSDVQITQSPSFLSASVGDRVTITCRASKSISKYLAWYQQKPGKANKLLIYSGSTLQSGVPSRFSGSGSGTDFTLTISSLQPEDFATYYCQQHNEYPWTFGGGTKVEIKRAAAGGGGSGGGGSHHHHHHHH

SEQ ID NO: 58 - protein, 264 aa, Artificial Sequence
  VH2-VL3 scFv
QVQLVQSGAEVKKPGASVKVSCKVSGYTFTDHTIHWMRQAPGQGLEWMGYNYPRDGSTKYNEKFQGRVTMTADKSTSTVYMELSSLRSEDTAVYYCAKGFITTVVPSAYWGQGTLVTVSSGGGGSGGGGSGGGGSDVQLTQSPSSVSASVGDRVTITCRASKSISKYLAWYQQKPGKAPKLLIYSGSTLQSGVPSRFSGSGSGTDFTLTISSLQPEDFATYYCQQHNEYPWTFGPGTKVEIKRAAAGGGGSGGGGSHHHHHHHH

SEQ ID NO: 59 - protein, 264 aa, Artificial Sequence
  VH3-VL1 scFv
QVQLVQSGAEVKKPGATVKISCKVSGYTFTDHTIHWMQQAPGKGLEWMGYNYPRDGSTKYNEKFQGRVTITADKSTSTAYMELSSLRSEDTAVYYCAKGFITTVVPSAYWGQGTLVTVSSGGGGSGGGGSGGGGSDIQLTQSPSFLSASVGDRVTITCRASKSISKYLAWYQQKPGKAPKLLIYSGSTLQSGVPSRFSGSGSGTEFTLTISSLQPEDFATYYCQQHNEYPWTFGGGTKVEIKRAAAGGGGSGGGGSHHHHHHHH

SEQ ID NO: 60 - protein, 264 aa, Artificial Sequence
  VH3-VL2 scFv
QVQLVQSGAEVKKPGATVKISCKVSGYTFTDHTIHWMQQAPGKGLEWMGYNYPRDGSTKYNEKFQGRVTITADKSTSTAYMELSSLRSEDTAVYYCAKGFITTVVPSAYWGQGTLVTVSSGGGGSGGGGSGGGGSDVQITQSPSFLSASVGDRVTITCRASKSISKYLAWYQQKPGKANKLLIYSGSTLQSGVPSRFSGSGSGTDFTLTISSLQPEDFATYYCQQHNEYPWTFGGGTKVEIKRAAAGGGGSGGGGSHHHHHHHH

SEQ ID NO: 61 - protein, 264 aa, Artificial Sequence
  VH3-VL3 scFv
QVQLVQSGAEVKKPGATVKISCKVSGYTFTDHTIHWMQQAPGKGLEWMGYNYPRDGSTKYNEKFQGRVTITADKSTSTAYMELSSLRSEDTAVYYCAKGFITTVVPSAYWGQGTLVTVSSGGGGSGGGGSGGGGSDVQLTQSPSSVSASVGDRVTITCRASKSISKYLAWYQQKPGKAPKLLIYSGSTLQSGVPSRFSGSGSGTDFTLTISSLQPEDFATYYCQQHNEYPWTFGPGTKVEIKRAAAGGGGSGGGGSHHHHHHHH

SEQ ID NO: 62 - protein, 271 aa, Artificial Sequence
  Mouse 6B5 scFv
MKKTAIAIAVALAGFATVAQAQVQLQQSDAELVKPGASVKISCKVSGYTFTDHTIHWMKQRPEQGLEWIGYNYPRDGSTKYNEKFKGKATLTADKSSSTAYMQLNSLTSEDSAVYFCAKGFITTVVPSAYWGQGTLVTVSAGGGGSGGGGSGGGGSDVQITQSPSYLAASPGETITINCRASKSISKYLAWYQEKPGKTNKLLIYSGSTLQSGIPSRFSGSGSGTDFTLTISSLEPEDFAMYYCQQHNEYPWTFGGGTKLEIKGSHHHHHH

SEQ ID NO: 63 - protein, 120 aa, Artificial Sequence
  Murine 6B5 VH parental
QVQLQQSDAELVKPGASVKISCKVSGYTFTDHTIHWMKQRPEQGLEWIGYNYPRDGSTKYNEKFKGKATLTADKSSSTAYMQLNSLTSEDSAVYFCAKGFITTVVPSAYWGQGTLVTVSA

SEQ ID NO: 64 - protein, 107 aa, Artificial Sequence
  Murine 6B5 VL parental
DVQITQSPSYLAASPGETITINCRASKSISKYLAWYQEKPGKTNKLLIYSGSTLQSGIPSRFSGSGSGTDFTLTISSLEPEDFAMYYCQQHNEYPWTFGGGTKLEIK

SEQ ID NO: 65 - DNA, 861 bp, Artificial Sequence
  VH3-VL3 scFv nucleic acid sequence
atgaagtaccttcttcccaccgccgcggctgggttgttgttacttgcagcacaaccggcgatggctcaagtccagttagttcagtcgggggccgaagtaaagaagccaggtgctactgtgaaaatttcgtgcaaagtgagcggatacacattcacggaccacacgattcactggatgcagcaagctccgggcaagggtcttgagtggatgggctacaactatccgcgtgacggatcaacaaaatacaatgaaaaatttcaagggcgtgttacaattaccgcggataaatccacgagtactgcctacatggagttgtcctcacttcgttcagaggacacagcagtgtactattgtgctaaagggttcatcacgaccgtggtcccctctgcttattggggccaaggaacacttgtgactgtgtcttctgggggcggggggagcggaggcggaggtagcggtggcgggggtagtgacgttcaactgactcaatcgccttcatccgttagcgccagcgtaggcgaccgtgtgaccatcacgtgccgcgcgtccaaaagtatcagcaagtacctggcctggtaccaacaaaaacccggaaaggcaccgaagttgttgatttattccggttcaacattacaaagcggcgttccgagtcgtttcagtggtagcggttccggcacagattttaccttgaccatttcctccctgcagccagaagactttgctacttattactgtcaacagcacaatgagtacccgtggacgtttgggcctggaactaaggttgagattaagcgtgctgctgccgggggcggtggttccggaggaggaggaagtcaccaccaccatcaccatcatcatggt

SEQ ID NO: 66 - DNA, 861 bp, Artificial Sequence
  VH3-VL2 scFv nucleic acid sequence
atgaaatatctgctgccaactgcggcagcaggtctgttgcttctggccgctcaaccggccatggctcaagtccagttagttcagagtggggcagaggttaaaaaaccgggagctacagtaaagatcagctgtaaagtatcaggttatacatttactgaccatactatccactggatgcaacaggcgccagggaaaggtttggagtggatgggatataattatccacgcgacgggtcaactaagtacaacgagaagtttcaaggccgtgtaacgattaccgcggacaaaagcacgagtacagcgtacatggaattatcatctttgcgctcggaggacacagcggtctattactgtgccaagggtttcatcactactgtggtaccaagtgcgtattggggtcaaggaacccttgttacggtgtcatcagggggtggcggaagtggcggtggtggatcgggcggaggtggaagcgatgttcagatcacacagtcgccctcgttcctgagtgcaagtgtcggtgatcgtgtgactattacgtgtcgtgcatcgaaatcaatctcaaagtatctggcttggtaccagcaaaaacctggaaaggctaacaaattgttgatctattccgggagcacccttcaaagcggtgtcccctctcgtttctccggatccgggtcagggaccgactttactctgactatttccagtcttcagccggaagattttgcgacttactattgccagcagcataatgagtacccatggacttttggcggtggcacaaaggtcgagattaagcgtgcagctgccggtggtggaggttcgggtgggggcggttctcatcatcaccatcatcaccatcatggt

SEQ ID NO: 67 - DNA, 861 bp, Artificial Sequence
  VH3-VL1 scFv nucleic acid sequence
atgaaatatttgcttccgactgccgccgcaggtctgttacttttagcagcgcagcccgctatggcacaggtccagttagttcaatcaggagcggaggtgaagaagccgggagccacggttaaaatctcatgcaaggtgtccggctatacatttaccgaccacacgattcactggatgcagcaagctcccgggaaggggcttgaatggatggggtacaattatccacgcgatggttccaccaagtataacgaaaaatttcaaggtcgtgtcaccattaccgctgacaaaagcacgtctacagcgtacatggagctgagtagcttgcgctcagaggacacagccgtatactattgcgcaaaaggtttcatcacgaccgtagtcccctctgcgtattggggacaggggaccctggtcacggtctcctccgggggcggaggatcgggaggcggggggtctggaggtggtggatctgacatccagcttacccaatcgcctagcttcttgagtgctagtgtaggcgaccgtgttactatcacttgtcgcgcttctaagagcattagcaaatacttagcctggtaccaacaaaagccgggaaaggcacccaagctgttaatttatagtgggtctacccttcagtccggcgtaccctcacgcttttccggcagtggctcgggtaccgaatttacccttacgatttcttcgcttcaacccgaagattttgcaacgtactactgtcagcagcacaacgagtatccctggacattcggcggagggacaaaagtagaaatcaagcgtgcagccgcaggtggcggcgggtctggcggcggagggagtcaccatcaccatcatcatcatcatgga

SEQ ID NO: 68 - DNA, 861 bp, Artificial Sequence
  VH2-VL3 scFv nucleic acid sequence
atgaaatatttgttacctaccgctgcggcaggacttctgcttttggccgctcagcccgcaatggctcaagtgcaattggttcagtcaggggccgaagtaaaaaagccaggcgcgagcgtaaaagtgagttgcaaggtctccggttacacgtttaccgatcacacgattcactggatgcgtcaagctccaggccagggtcttgaatggatgggttacaactatcctcgcgatggttcgaccaagtataacgagaagtttcagggccgtgtcacaatgaccgccgacaaatcaacgagcactgtctacatggagctgtcatccctgcgcagcgaggatacagctgtgtactactgtgccaagggcttcattactaccgtcgtccccagcgcgtactggggtcaaggtacactggtaacagtttcatccggaggagggggaagcggcggcggtggatctggcggcggtgggtcagacgttcaacttacccagtcgccttcttccgtgagtgcctctgtcggggatcgtgttaccatcacttgccgcgcatctaagtcaatttctaaatatttggcctggtatcagcagaaacccggtaaagcgcccaaattgttgatctattccggcagtaccttgcaatccggggtgccttcgcgcttctcggggagtggaagcggcacggatttcactttaacgatctcgagtttgcagccggaagattttgcgacttactattgtcagcagcataacgaatatccatggacctttggccctggtacgaaagtagaaatcaaacgtgcagcagccggtgggggtggctccggtggcggtgggtcgcatcaccaccaccatcatcatcacggt

SEQ ID NO: 69 - DNA, 861 bp, Artificial Sequence
  VH2-VL2 scFv nucleic acid sequence
atgaagtacctgttgcccacagccgctgctgggttactgcttcttgctgcccagcccgcaatggcgcaagtgcaattagtccagtctggagcagaggttaaaaagccgggagcttcagtgaaggtctcctgtaaggtaagtggttatacattcaccgatcacacaatccattggatgcgccaggccccaggtcagggtcttgaatggatgggctataactacccgcgtgatggctcaactaagtataacgagaagtttcaggggcgcgttacaatgactgcggataaaagcacgtcgacggtgtacatggaattgtcaagccttcgttccgaagataccgcagtttactattgtgctaagggctttatcactaccgtggtacccagtgcgtactgggggcagggaaccctggtaaccgtgtcatcgggcggaggcggaagcgggggaggtggcagtggaggtggcgggtctgacgttcaaatcacccagtcaccgtcatttctttccgcgtctgtgggtgaccgcgtaacaattacttgccgtgcttcgaaaagcatttcgaaataccttgcctggtaccaacagaaaccggggaaagcaaacaaacttttaatctacagcgggagcacgcttcaatccggcgtcccatcccgtttttctggctccggcagcgggaccgacttcaccttaactatttcttcccttcaaccggaggactttgcgacgtattactgtcaacaacacaatgagtatccgtggactttcggaggcggaactaaggttgaaatcaagcgtgctgctgctggcgggggaggctcaggcggagggggatcacatcatcatcaccatcatcatcacgga

SEQ ID NO: 70 - DNA, 861 bp, Artificial Sequence
  VH2-VL1 scFv nucleic acid sequence
atgaaatacttgctgccgactgccgcagcgggattattattacttgcggctcagccggctatggcgcaggtccagttagttcagagtggggcagaagtgaagaaacccggtgcatctgtaaaggtctcatgtaaagtatctggctacaccttcactgaccacactatccactggatgcgtcaagcaccaggacaaggtttagagtggatgggatataactatccgcgtgacgggagtacgaagtataacgaaaaatttcagggccgtgtaaccatgaccgcggataaatccacttccactgtctatatggaattatcgtcgttacgtagcgaggacacggcggtatattattgcgccaaagggtttatcacgactgttgtgccgtccgcttactgggggcaagggactttagtgaccgtgtccagcggaggggggggtagcgggggtggcgggagtggtggtgggggttcggacattcagcttacccaatcccctagctttttgtcagcctccgttggcgatcgtgtaactattacgtgccgcgcctccaagtccatttcaaaatatttagcctggtaccaacagaagccaggaaaagctcctaaattactgatttactcaggttccacattgcagtcgggcgtaccaagccgtttttcgggaagtggtagcgggaccgagtttacattgacgattagtagtcttcaaccggaggattttgcaacctactattgtcagcagcacaacgagtacccatggacctttggaggcggtaccaaagtggaaattaaacgcgcagcagcaggcggcggtggttcagggggaggaggctcgcatcaccaccatcatcatcaccacggt

SEQ ID NO: 71 - DNA, 861 bp, Artificial Sequence
  VH1-VL3 scFv nucleic acid sequence
atgaaataccttttgccgactgccgccgcaggattattgttactggcggctcagccggctatggcccaagtccaattagttcaatcaggggcagaagttaagaagcccggagcaagtgtcaaggtctcatgcaaagcctccggttacacctttaccgaccacacgatgcactgggttcgccaagctcccggacagggcctggaatggatgggttataattatccgcgtgatggtagcacgaaatacgcggaaaaattccaaggtcgcgttacgatgaccgcggacaagtctactagcaccgtgtacatggaacttagctcgctgcgttcggaagatacggcggtgtactactgtgcgaaaggtttcatcactacagtagtgccaagtgcgtattggggtcaaggcacgctggtaacggtttcaagtggtggcggcggtagcggcggcggcggcagcggaggagggggatcggatgtccaacttacgcaatctccgtcctctgtttccgcaagtgtgggcgaccgcgtaaccatcacttgccgtgctagtaaaagcatttctaagtatttagcgtggtatcaacagaagcccggaaaggcgccaaagctgttgatttattccgggagtacattacaatctggcgtgccgtcccgcttctccggcagcggtagtggtactgacttcacgctgacaattagttcacttcagccagaggattttgcgacatattattgccagcagcataacgaatacccatggaccttcggtcctggaaccaaggttgaaatcaaacgtgctgcggccggcggcggtgggagcggagggggcgggtcacatcatcatcatcatcaccatcatggt

SEQ ID NO: 72 - DNA, 861 bp, Artificial Sequence
  VH1-VL2 scFv nucleic acid sequence
atgaaataccttcttcccaccgcagcagcgggattgttattattggctgcacaacctgcgatggctcaagtacagttggtgcagtcaggggcggaagtcaagaaaccaggcgcttcagtgaaagtttcgtgtaaagcatccggctatacttttaccgaccacaccatgcactgggttcgccaagctcctggacagggtctggaatggatggggtacaactatccccgcgatggatccacaaagtacgcggagaagttccaaggacgtgtaacaatgacggccgataaaagcacttccacagtctatatggaactttcgtctcttcgttctgaggacacagcagtttactactgtgctaaaggatttatcactaccgtcgttccgtctgcatattgggggcagggcacgttagtaacagtcagctccgggggcgggggctcagggggcggtggatcagggggaggcggctctgacgtgcagatcactcagtcgcctagctttctttcggctagtgtcggggatcgcgtcactatcacatgccgcgccagcaaaagcatctctaaatacctggcttggtaccaacaaaaacccggaaaggctaataagttgctgatctacagtgggagtactttgcagtcgggggtgccgagtcgtttttcaggtagcgggtcgggcacggactttacccttacaatttcctccctgcagcccgaggactttgccacatattattgtcaacagcacaacgagtacccgtggacgtttgggggaggtaccaaagtggaaatcaagcgtgcagcggccgggggaggtggaagcggcggcggtggaagtcaccatcatcaccaccaccatcacgga

SEQ ID NO: 73 - DNA, 861 bp, Artificial Sequence
  VH1-VL1 scFv nucleic acid sequence
atgaaatacctgttacctactgctgccgcaggtttgttgcttctggcggctcaaccggccatggcacaggttcagctggtgcaatcaggcgccgaagtcaaaaaaccgggtgcaagcgtcaaggtgagctgtaaggcaagcggatatacttttacagatcatacaatgcactgggtacgccaggcaccaggccagggccttgaatggatgggatataactacccacgtgatggatctactaaatatgccgagaagttccagggtcgcgttaccatgactgctgataaaagtacatcaactgtatacatggaacttagctcattgcgttccgaagatactgccgtgtactattgtgcaaaggggtttatcacgacagtcgttccatcggcatattggggccagggaacgttagtaacagtcagcagtgggggtggggggtcaggcggaggagggtctggtggggggggttctgacatccagttgacacagtccccatcctttttgtctgcatcggttggggaccgcgtgacgattacttgtcgcgcgtccaagtctatcagcaaatatttagcatggtatcaacaaaaacctggcaaggctcccaagttacttatttactccggtagtactcttcagtcgggagtgccttcccgttttagcgggtctggttcaggcacggagtttacccttacaattagttctctgcagcccgaggattttgcaacttactactgccagcaacacaatgagtacccctggacattcggcggtgggacaaaagtcgagattaagcgtgccgctgccggtggaggagggtcagggggtggcggcagtcatcaccaccatcaccatcatcatgga

SEQ ID NO: 74 - DNA, 861 bp, Artificial Sequence
  6B5 scFv nucleic acid sequence
atgaagtacttattgcccactgctgctgctggattattattgttggcagcgcaaccggccatggcgcaggtccaacttcagcagtcagatgccgaacttgtaaagccgggtgcaagcgtgaaaatctcatgtaaagtatctggttatacgtttacagatcacaccatccactggatgaagcaacgccctgagcagggtttagagtggattggctataattatccgcgcgacggttcgacaaaatacaacgaaaagttcaagggcaaggcaacgcttaccgccgataagagttcaagtacagcatatatgcaactgaacagcttaactagcgaagatagcgcagtttacttttgcgcgaagggatttatcaccaccgtggttccgagtgcctactggggacagggcacattggttacagtcagtgcaggaggaggagggtccggtggcggaggatcgggtgggggtggatcagatgtccaaatcacacaatcgccatcctacttggccgcctcgcccggagaaaccatcactattaattgccgcgcgagcaagtctatttccaagtatttggcatggtaccaagaaaagcccggtaaaactaacaaacttttgatctactctgggtccacgctgcagtcaggaatcccatcccgtttctcgggcagcggatctgggacagacttcacgttgacaatttcgagccttgagccggaagatttcgcaatgtactactgtcagcaacataacgagtacccttggacatttggcgggggcacaaagcttgaaattaaacgcgctgctgccggaggaggtggttcggggggagggggttctcatcatcaccaccatcaccaccacgga

SEQ ID NO: 75 - protein, 19 aa, Artificial Sequence
  Signal sequence
MEWSWVFLFFLSVTTGVHS

SEQ ID NO: 76 - protein, 22 aa, Artificial Sequence
  C-terminal tag
RAAAGGGGSGGGGSHHHHHHHH